European Patent Application EP 4 219 446 A2, published August 2, 2023. Title: Traceless Reductively Cleavable Linker molecules for Peptide Purification. Applicant: Gyros Protein Technologies AB. The sequence listing filed with the application follows.

SEQUENCE LISTING (6 sequences)

SEQ ID NO: 1 - protein, 15 aa, synthetic construct
  REGION 1..15: note = fragment 2-16 of the Histone H3 protein
ARTKQTARKSTGGKA

SEQ ID NO: 2 - protein, 13 aa, synthetic construct
  REGION 1..13: note = test peptide
AKADEVSLHKWYG

SEQ ID NO: 3 - protein, 15 aa, synthetic construct
  REGION 1..15: note = fragment 81-95 of the human cytomegalovirus lower matrix phosphoprotein (CMV)
YFTGSEVENVSVNVH

SEQ ID NO: 4 - protein, 11 aa, synthetic construct
  REGION 1..11: note = fragment 510-520 of humane Lemur Tyrosine Kinase 3 (LMTK3)
PSNPFYEALST

SEQ ID NO: 5 - protein, 20 aa, synthetic construct
  REGION 1..20: note = fragment 1-20 of humane amyloid beta
DAEFRHDSGYEVHHQKLVFF

SEQ ID NO: 6 - protein, 13 aa, synthetic construct
  REGION 1..13: note = test peptide
CKADEVSMHKWYG